European Patent Application EP 4 410 819 A1, published August 7, 2024. Title: Peptide having anti-inflammatory activity and use thereof. Applicant: CAREGEN CO., LTD. The sequence listing filed with the application follows.

SEQUENCE LISTING (15 sequences)

SEQ ID NO: 1 - protein, 12 aa, synthetic construct
  REGION 1..12: note = peptide
SVSVGMKPSPRP

SEQ ID NO: 2 - DNA, 20 bp, synthetic construct
  misc_feature 1..20: note = COX2-F
  source 1..20: mol_type = other DNA
tgagtggtagccagcaaagc

SEQ ID NO: 3 - DNA, 20 bp, synthetic construct
  misc_feature 1..20: note = COX2-R
  source 1..20: mol_type = other DNA
ctgcagtccaggttcaatgg

SEQ ID NO: 4 - DNA, 20 bp, synthetic construct
  misc_feature 1..20: note = INF gamma-F
  source 1..20: mol_type = other DNA
gaggtcaacaacccacaggt

SEQ ID NO: 5 - DNA, 20 bp, synthetic construct
  misc_feature 1..20: note = INF gamma-R
  source 1..20: mol_type = other DNA
gggacaatctcttccccacc

SEQ ID NO: 6 - DNA, 21 bp, synthetic construct
  misc_feature 1..21: note = TNF alpha-F
  source 1..21: mol_type = other DNA
aacatccaaccttcccaaacg

SEQ ID NO: 7 - DNA, 21 bp, synthetic construct
  misc_feature 1..21: note = TNF alpha-R
  source 1..21: mol_type = other DNA
gaccctaagcccccaattctc

SEQ ID NO: 8 - DNA, 21 bp, synthetic construct
  misc_feature 1..21: note = COX2-F
  source 1..21: mol_type = other DNA
atcattcaccaggcaaattgc

SEQ ID NO: 9 - DNA, 21 bp, synthetic construct
  misc_feature 1..21: note = COX2-R
  source 1..21: mol_type = other DNA
ggcttcagcataaagcgtttg

SEQ ID NO: 10 - DNA, 20 bp, synthetic construct
  misc_feature 1..20: note = IL-6-F
  source 1..20: mol_type = other DNA
aaagaggcactgccagaaaa

SEQ ID NO: 11 - DNA, 20 bp, synthetic construct
  misc_feature 1..20: note = IL-6-R
  source 1..20: mol_type = other DNA
atctgaggtgcccatgctac

SEQ ID NO: 12 - DNA, 20 bp, synthetic construct
  misc_feature 1..20: note = IL-8-F
  source 1..20: mol_type = other DNA
gaaggtgcagttttgccaag

SEQ ID NO: 13 - DNA, 20 bp, synthetic construct
  misc_feature 1..20: note = IL-8-R
  source 1..20: mol_type = other DNA
accctctgcacccagttttc

SEQ ID NO: 14 - DNA, 20 bp, synthetic construct
  misc_feature 1..20: note = GAPDH-F
  source 1..20: mol_type = other DNA
ggagccaaaagggtcatcat

SEQ ID NO: 15 - DNA, 20 bp, synthetic construct
  misc_feature 1..20: note = GAPDH-R
  source 1..20: mol_type = other DNA
gtgatggcatggactgtggt